European Patent Application EP 4 414 460 A1, published August 14, 2024. Title: Compositions comprising a sequence specific endoribonuclease and methods of use. Applicant: Arcticzymes AS. Application EP. The sequence listing filed with the application follows.

SEQUENCE LISTING (12 sequences)

SEQ ID NO: 1 - protein, 176 aa, Escherichia coli
MAKFFTISSSYIKYLKDFDDKVPNSEDPTYNNPKAFIGIVLEIEGHKYLAPLTSPKAWHANVKESSPAFFKLHENGVPDNQLGLINLKFMIPIIEAEVSLLDLDSMPDTPYKRMLYKQLQFIRVNEDKISEKSKLLRNLALQGRMQGTCDFAVLEEKYQHFGKKPEDMEIDDLESR

SEQ ID NO: 2 - protein, 187 aa, Escherichia coli
MNHKVHHHHHHMAKFFTISSSYIKYLKDFDDKVPNSEDPTYNNPKAFIGIVLEIEGHKYLAPLTSPKAWHANVKESSPAFFKLHENGVPDNQLGLINLKFMIPIIEAEVSLLDLDSMPDTPYKRMLYKQLQFIRVNEDKISEKSKLLRNLALQGRMQGTCDFAVLEEKYQHFGKKPEDMEIDDLESR

SEQ ID NO: 3 - DNA, 516 bp, Escherichia coli
  source 1..516: mol_type = genomic DNA
atgaaatttttcacaatatcaagcagttacataaaatacctgaaggactttgatgacaaagttcccaatagcgaagatcctacatacaacaatcctaaggctttcattggcatagtactagagattgaaggacataaatatttagcacctttaacatcgccaaaagcatggcatgctaatgtaaaagagtcatcacccgccttcttcaaacttcatgaaaacggtgtccctgataatcagcttggattgattaatctgaaatttatgattccaataatcgaagctgaagtgtctttacttgatctggatagcatgcctgatacgccttacaaaagaatgctatataaacagttacaatttattcgtgtaaatgaagataaaatatctgaaaaatcaaaactattaagaaaccttgccttgcaaggcagaatgcaaggaacatgcgactttgccgtgttagaagaaaaatatcaacatttcggtaaaaaacctgaagacatggaaatagacgattaa

SEQ ID NO: 4 - DNA, 166 bp, Escherichia coli
  source 1..166: mol_type = genomic DNA
aggtgatttgctacctttaagtgcagctagaaatttaggtgatttgctacctttaagtgcagctagaaatttaggtgatttgctacctttaagtgcagctagaaattcaggtgatttgctacctttaagtgcagctagaaatttaggtcatttactaccttaaagt

SEQ ID NO: 5 - RNA, 36 nt, Escherichia coli
  source 1..36: mol_type = transcribed RNA
attcaggtgatttgctacctttaagtgcagctagaa

SEQ ID NO: 6 - protein, 171 aa, Pectobacterium atrosepticum
MKFYTISSKYIEYLKEFDDKVPNSEDPTYQNPKAFIGIVLEIQGHKYLAPLTSPKKWHNNVKESSLSCFKLHENGVPENQLGLINLKFMIPIIEAEVSLLDLGNMPNTPYKRMLYKQLQFIRANSDKIASKSDTLRNLVLQGKMQGTCNFSLLEEKYRDFGKEAEDTEEGE

SEQ ID NO: 7 - protein, 194 aa, Bacillus thuringiensis
MTNKDNPKFHTISTEYIDYLREADSKVPFNKDEQHSRPYVGVLEKINGHDYFVPLTSRNDKNFNSQVSVKLFDNDEKRIGVLLVNNMIPVPEKECKEIDIAEKTAADPQYGNLMLKQYLFLKENMDRVTNKVEKVYKDVTVQGKPSHKQKFLKGVCCDFPKLEEKCQEYKERDQAKERDKARRIAYMRQMGRER

SEQ ID NO: 8 - protein, 183 aa, Lactococcus lactis
MSSFFYKEILRMTLRFFTVTDEYIAYLRKFESKVHYQYENNASTYVGVVLKKNDFNYFIPLSSYKKGNPEKDKAMKKRSRIVTRLFEIGNINNPLGYLLHHNMIPVPDSELIPLPLDLKKPKHKMMQKQLIYMKSISEKIENKSEVVYRKAAHEKDGYYLKFSCDFKLLEAKATLYSKKSTFQ

SEQ ID NO: 9 - protein, 162 aa, Eubacterium rectale
MIRNGFYIIKDRFFSDMSDPYLKGNKKQNRPHYYCFEDSNYNGIYWMIPLSSRIDKYKKIVSKRTGKGRNCDIIHIVKLDDSHESAFLIQDMFPISDKYIEREYTIAGNHLRLTSEHAAKEIEQKARKVLGMLKRGIKFTPTQPDIQKIYERLQQDLPATHL

SEQ ID NO: 10 - RNA, 50 nt, synthetic construct
  source 1..50: mol_type = other RNA
cgcaattgccgcattacaagggaaataacttcgtacgttgttgttagcat

SEQ ID NO: 11 - DNA, 31 bp, synthetic construct
  source 1..31: mol_type = other DNA
aggtcatatggcgaaatttttcacaatatca

SEQ ID NO: 12 - DNA, 29 bp, synthetic construct
  source 1..29: mol_type = other DNA
ggaaatagacgatctcgagtctagagcat